European Patent Application EP 4 721 762 A2, published April 8, 2026. Title: MODIFIED POLYAMINE POLYMERS FOR DELIVERY OF BIOMOLECULES INTO CELLS. Applicant: Promega Corporation. Application EP. The sequence listing filed with the application follows.

SEQUENCE LISTING (12 sequences)

SEQ ID NO: 1 - protein, 170 aa, synthetic construct
  REGION 1..170: note = synthetic
MFTLADFVGDWQQTAGYNQDQVLEQGGLSSLFQALGVSVTPIQKVVLSGENGLKADIHVIIPYEGLSGFQMGLIEMIFKVVYPVDDHHFKIILHYGTLVIDGVTPNMIDYFGRPYPGIAVFDGKQITVTGTLWNGNKIYDERLINPDGSLLFRVTINGVTGWRLCENILA

SEQ ID NO: 2 - protein, 171 aa, synthetic construct
  REGION 1..171: note = synthetic
MVFTLEDFVGDWRQTAGYNLDQVLEQGGVSSLFQNLGVSVTPIQRIVLSGENGLKIDIHVIIPYEGLSGDQMGQIEKIFKVVYPVDDHHFKVILHYGTLVIDGVTPNMIDYFGRPYEGIAVFDGKKITVTGTLWNGNKIIDERLINPDGSLLFRVTINGVTGWRLCERILA

SEQ ID NO: 3 - protein, 11 aa, synthetic construct
  REGION 1..11: note = synthetic
VSGWRLFKKIS

SEQ ID NO: 4 - protein, 158 aa, synthetic construct
  REGION 1..158: note = synthetic
MVFTLEDFVGDWRQTAGYNLDQVLEQGGVSSLFQNLGVSVTPIQRIVLSGENGLKIDIHVIIPYEGLSGDQMGQIEKIFKVVYPVDDHHFKVILHYGTLVIDGVTPNMIDYFGRPYEGIAVFDGKKITVTGTLWNGNKIIDERLINPDGSLLFRVTIN

SEQ ID NO: 5 - protein, 11 aa, synthetic construct
  REGION 1..11: note = synthetic
VTGYRLFEEIL

SEQ ID NO: 6 - protein, 11 aa, synthetic construct
  REGION 1..11: note = synthetic
VSGWALFKKIS

SEQ ID NO: 7 - protein, 12 aa, synthetic construct
  REGION 1..12: note = synthetic
MVSGWALFKKIS

SEQ ID NO: 8 - protein, 14 aa, synthetic construct
  REGION 1..14: note = synthetic
MGVTGWRLCERILA

SEQ ID NO: 9 - protein, 147 aa, synthetic construct
  REGION 1..147: note = synthetic
VFTLDDFVGDWEQTAAYNLDQVLEQGGVSSLLQNLAVSVTPIMRIVRSGENALKIDIHVIIPYEGLSADQMAQIEEVFKVVYPVDDHHFKVILPYGTLVIDGVTPNKLNYFGRPYEGIAVFDGKKITVTGTLWNGNKIIDERLITPD

SEQ ID NO: 10 - protein, 147 aa, synthetic construct
  REGION 1..147: note = synthetic
VFTLDDFVGDWEQTAAYNLDQVLEQGGVSSLLQNLAVSVTPIMRIVRSGENALKIDIHVIIPYEGLSADQMAQIEEVFKVVYPVDDHHFKVILPYGTLVIDGVTPNKLNYFGRPYEGIAVFDGKKITTTGTLWNGNKIIDERLITPD

SEQ ID NO: 11 - protein, 147 aa, synthetic construct; identical to SEQ ID NO: 10
  REGION 1..147: note = synthetic

SEQ ID NO: 12 - protein, 11 aa, synthetic construct
  REGION 1..11: note = synthetic
GSMLFRVTINS